European Patent Application EP 4 737 902 A1, published May 6, 2026. Title: 파킨슨병 진단용 조성물 및 이를 이용한 파킨슨병 진단 방법. Applicant: Research ＆ Business Foundation SUNGKYUNKWAN UNIVERSITY. Application KR. The sequence listing filed with the application follows.

SEQUENCE LISTING (41 sequences)

SEQ ID NO: 1 - DNA, 22 bp, synthetic construct
  source 1..22: mol_type = other DNA
aagcagtggtatcaacgcagag

SEQ ID NO: 2 - DNA, 24 bp, synthetic construct
  source 1..24: mol_type = other DNA
acattgatgtctttggggtagaag

SEQ ID NO: 3 - DNA, 20 bp, synthetic construct
  source 1..20: mol_type = other DNA
atcgtacacaccagtgtggc

SEQ ID NO: 4 - DNA, 20 bp, synthetic construct
  source 1..20: mol_type = other DNA
gggatccagagttccaggtc

SEQ ID NO: 5 - protein, 8 aa, synthetic construct
GFTFSDFY

SEQ ID NO: 6 - protein, 10 aa, synthetic construct
SRNKANDYTT

SEQ ID NO: 7 - protein, 13 aa, synthetic construct
ARDAFYGYGAMDY

SEQ ID NO: 8 - protein, 6 aa, synthetic construct
KSIRKY

SEQ ID NO: 9 - skipped

SEQ ID NO: 10 - protein, 9 aa, synthetic construct
QQHNEYPYT

SEQ ID NO: 11 - protein, 141 aa, synthetic construct
MKLWLNWVFLLTLLHGIQCEVKLVESGGGLVQPGGSLRLSCATSGFTFSDFYMEWVRQPPGKRLEWIAASRNKANDYTTEYSESVKGRFIVSRDISQSILYLQMNALRAEDTAIYYCARDAFYGYGAMDYWGQGTSVTVSS

SEQ ID NO: 12 - protein, 139 aa, synthetic construct
MGNQFLPGHSLDMRFQVQVLGLLLLWISGAQCDVQITQSPSYLAASPGETITINCRASKSIRKYLAWYQEKPGKTNKLLIYSGSTLQSGIPSRFSGSGSGTDFTLTISSLEPEDFAMYYCQQHNEYPYTFGGGTKLEIK

SEQ ID NO: 13 - protein, 127 aa, synthetic construct
MRFQVQVLGLLLLWISGAQCDVQITQSPSYLAASPGETITINCRASKSIRKYLAWYQEKPGKTNKLLIYSGSTLQSGIPSRFSGSGSGIDFTLTISSLEPEDFAMYYCQQHNEYPYTFGGGTKLEIK

SEQ ID NO: 14 - protein, 467 aa, synthetic construct
MKLWLNWVFLLTLLHGIQCEVKLVESGGGLVQPGGSLRLSCATSGFTFSDFYMEWVRQPPGKRLEWIAASRNKANDYTTEYSESVKGRFIVSRDISQSILYLQMNALRAEDTAIYYCARDAFYGYGAMDYWGQGTSVTVSSASTKGPSVFPLAPCSRSTSESTAALGCLVKDYFPEPVTVSWNSGALTSGVHTFPAVLQSSGLYSLSSVVTVPSSNFGTQTYTCNVDHKPSNTKVDKTVERKCCVECPPCPAPPVAGPSVFLFPPKPKDTLMISRTPEVTCVVVDVSHEDPEVQFNWYVDGVEVHNAKTKPREEQFNSTFRVVSVLTVVHQDWLNGKEYKCKVSNKGLPAPIEKTISKTKGQPREPQVYTLPPSREEMTKNQVSLTCLVKGFYPSDISVEWESNGQPENNYKTTPPMLDSDGSFFLYSKLTVDKSRWQQGNVFSCSVMHEALHNHYTQKSLSLSPGK

SEQ ID NO: 15 - protein, 246 aa, synthetic construct
MGNQFLPGHSLDMRFQVQVLGLLLLWISGAQCDVQITQSPSYLAASPGETITINCRASKSIRKYLAWYQEKPGKTNKLLIYSGSTLQSGIPSRFSGSGSGTDFTLTISSLEPEDFAMYYCQQHNEYPYTFGGGTKLEIKRTVAAPSVFIFPPSDEQLKSGTASVVCLLNNFYPREAKVQWKVDNALQSGNSQESVTEQDSKDSTYSLSSTLTLSKADYEKHKVYACEVTHQGLSSPVTKSFNRGEC

SEQ ID NO: 16 - protein, 234 aa, synthetic construct
MRFQVQVLGLLLLWISGAQCDVQITQSPSYLAASPGETITINCRASKSIRKYLAWYQEKPGKTNKLLIYSGSTLQSGIPSRFSGSGSGIDFTLTISSLEPEDFAMYYCQQHNEYPYTFGGGTKLEIKRTVAAPSVFIFPPSDEQLKSGTASVVCLLNNFYPREAKVQWKVDNALQSGNSQESVTEQDSKDSTYSLSSTLTLSKADYEKHKVYACEVTHQGLSSPVTKSFNRGEC

SEQ ID NO: 17 - protein, 10 aa, synthetic construct
GFSLSTSGMG

SEQ ID NO: 18 - protein, 7 aa, synthetic construct
IWWDDDK

SEQ ID NO: 19 - protein, 10 aa, synthetic construct
ARIANSWFAY

SEQ ID NO: 20 - protein, 10 aa, synthetic construct
KSVSTSAYSY

SEQ ID NO: 21 - protein, 10 aa, synthetic construct
KSVSTSGYTY

SEQ ID NO: 22 - skipped

SEQ ID NO: 23 - protein, 9 aa, synthetic construct
QHSRELPPT

SEQ ID NO: 24 - protein, 137 aa, synthetic construct
MGRLTSSFLLLIVPAYVLSQVTLKESGPGILQPSQTLSLTCSFSGFSLSTSGMGVGWIRQPSGKGLEWLAHIWWDDDKYYNTALKSGLTISKDTSKNQVFLKIASVDTADTATYYCARIANSWFAYWGQGTLVTVSA

SEQ ID NO: 25 - protein, 144 aa, synthetic construct
MGDKCAVMGRLTSSFLLLIVPAYVLSQVTLKESGPGILQPSQTLSLTCSFSGFSLSTSGMGVGWIRQPSGKGLEWLAHIWWDDDKYYNTALKSGLTISKDTSKNQVFLKIASVDTADTATYYCARIANSWFAYWGQGTLVTVSA

SEQ ID NO: 26 - protein, 148 aa, synthetic construct
MGSCQEPKKHPLFQLSEMETDTLLLWVLLLWVPGSTGDIVLTQSPASLAVSLGQRATISCRASKSVSTSAYSYMHWYQQKPGQPPKLLIYLASNLDSGVPARFSGSGSGTDFTLNIHPVEEEDAATYYCQHSRELPPTFGAGTKLELK

SEQ ID NO: 27 - protein, 131 aa, synthetic construct
METDTLLLWVLLLWVPGSTGDIVLTQSPASLAVSLGQRATISCRASKSVSTSGYTYMHWYQQKPGQSPKLLIYLASNLESGVPARFSGSGSGTDFTLNIHPVEEEDAATYYCQHSRELPPTFGAGTKLELK

SEQ ID NO: 28 - protein, 463 aa, synthetic construct
MGRLTSSFLLLIVPAYVLSQVTLKESGPGILQPSQTLSLTCSFSGFSLSTSGMGVGWIRQPSGKGLEWLAHIWWDDDKYYNTALKSGLTISKDTSKNQVFLKIASVDTADTATYYCARIANSWFAYWGQGTLVTVSAASTKGPSVFPLAPCSRSTSESTAALGCLVKDYFPEPVTVSWNSGALTSGVHTFPAVLQSSGLYSLSSVVTVPSSNFGTQTYTCNVDHKPSNTKVDKTVERKCCVECPPCPAPPVAGPSVFLFPPKPKDTLMISRTPEVTCVVVDVSHEDPEVQFNWYVDGVEVHNAKTKPREEQFNSTFRVVSVLTVVHQDWLNGKEYKCKVSNKGLPAPIEKTISKTKGQPREPQVYTLPPSREEMTKNQVSLTCLVKGFYPSDISVEWESNGQPENNYKTTPPMLDSDGSFFLYSKLTVDKSRWQQGNVFSCSVMHEALHNHYTQKSLSLSPGK

SEQ ID NO: 29 - protein, 470 aa, synthetic construct
MGDKCAVMGRLTSSFLLLIVPAYVLSQVTLKESGPGILQPSQTLSLTCSFSGFSLSTSGMGVGWIRQPSGKGLEWLAHIWWDDDKYYNTALKSGLTISKDTSKNQVFLKIASVDTADTATYYCARIANSWFAYWGQGTLVTVSAASTKGPSVFPLAPCSRSTSESTAALGCLVKDYFPEPVTVSWNSGALTSGVHTFPAVLQSSGLYSLSSVVTVPSSNFGTQTYTCNVDHKPSNTKVDKTVERKCCVECPPCPAPPVAGPSVFLFPPKPKDTLMISRTPEVTCVVVDVSHEDPEVQFNWYVDGVEVHNAKTKPREEQFNSTFRVVSVLTVVHQDWLNGKEYKCKVSNKGLPAPIEKTISKTKGQPREPQVYTLPPSREEMTKNQVSLTCLVKGFYPSDISVEWESNGQPENNYKTTPPMLDSDGSFFLYSKLTVDKSRWQQGNVFSCSVMHEALHNHYTQKSLSLSPGK

SEQ ID NO: 30 - protein, 255 aa, synthetic construct
MGSCQEPKKHPLFQLSEMETDTLLLWVLLLWVPGSTGDIVLTQSPASLAVSLGQRATISCRASKSVSTSAYSYMHWYQQKPGQPPKLLIYLASNLDSGVPARFSGSGSGTDFTLNIHPVEEEDAATYYCQHSRELPPTFGAGTKLELKRTVAAPSVFIFPPSDEQLKSGTASVVCLLNNFYPREAKVQWKVDNALQSGNSQESVTEQDSKDSTYSLSSTLTLSKADYEKHKVYACEVTHQGLSSPVTKSFNRGEC

SEQ ID NO: 31 - protein, 238 aa, synthetic construct
METDTLLLWVLLLWVPGSTGDIVLTQSPASLAVSLGQRATISCRASKSVSTSGYTYMHWYQQKPGQSPKLLIYLASNLESGVPARFSGSGSGTDFTLNIHPVEEEDAATYYCQHSRELPPTFGAGTKLELKRTVAAPSVFIFPPSDEQLKSGTASVVCLLNNFYPREAKVQWKVDNALQSGNSQESVTEQDSKDSTYSLSSTLTLSKADYEKHKVYACEVTHQGLSSPVTKSFNRGEC

SEQ ID NO: 32 - protein, 9 aa, synthetic construct
DYSITSGYS

SEQ ID NO: 33 - protein, 7 aa, synthetic construct
IHYRGST

SEQ ID NO: 34 - protein, 9 aa, unidentified
ATWDYRLAY

SEQ ID NO: 35 - protein, 7 aa, synthetic construct
SQHSTYT

SEQ ID NO: 36 - protein, 7 aa, synthetic construct
LKKDGSH

SEQ ID NO: 37 - protein, 13 aa, synthetic construct
GVGDTIKEQFVYV

SEQ ID NO: 38 - protein, 134 aa, synthetic construct
MRVLILLCLFTAFPGILSDVQLQESGPDLVKPSQSLSLTCTVTDYSITSGYSWHWIRQFPGNKLEWMAYIHYRGSTNYNPSLKSRISITRDTSKNQFFLQLNSVTTEDTATYYCATWDYRLAYWGQGTLVTVSA

SEQ ID NO: 39 - protein, 149 aa, synthetic construct
MGNLSVSAEISSTCIMAWTPLFFFFVLHCSGSFSQLVLTQSSSASFSLGASAKLTCTLSSQHSTYTIEWYQQQPLKPPKYVMELKKDGSHSTGDGIPDRFSGSSSGADRYLSISNIQPEDEAIYICGVGDTIKEQFVYVFGGGTKVTVL

SEQ ID NO: 40 - protein, 460 aa, synthetic construct
MRVLILLCLFTAFPGILSDVQLQESGPDLVKPSQSLSLTCTVTDYSITSGYSWHWIRQFPGNKLEWMAYIHYRGSTNYNPSLKSRISITRDTSKNQFFLQLNSVTTEDTATYYCATWDYRLAYWGQGTLVTVSAASTKGPSVFPLAPCSRSTSESTAALGCLVKDYFPEPVTVSWNSGALTSGVHTFPAVLQSSGLYSLSSVVTVPSSNFGTQTYTCNVDHKPSNTKVDKTVERKCCVECPPCPAPPVAGPSVFLFPPKPKDTLMISRTPEVTCVVVDVSHEDPEVQFNWYVDGVEVHNAKTKPREEQFNSTFRVVSVLTVVHQDWLNGKEYKCKVSNKGLPAPIEKTISKTKGQPREPQVYTLPPSREEMTKNQVSLTCLVKGFYPSDISVEWESNGQPENNYKTTPPMLDSDGSFFLYSKLTVDKSRWQQGNVFSCSVMHEALHNHYTQKSLSLSPGK

SEQ ID NO: 41 - protein, 255 aa, synthetic construct
MGNLSVSAEISSTCIMAWTPLFFFFVLHCSGSFSQLVLTQSSSASFSLGASAKLTCTLSSQHSTYTIEWYQQQPLKPPKYVMELKKDGSHSTGDGIPDRFSGSSSGADRYLSISNIQPEDEAIYICGVGDTIKEQFVYVFGGGTKVTVLGQPKAAPSVTLFPPSSEELQANKATLVCLISDFYPGAVTVAWKADSSPVKAGVETTTPSKQSNNKYAASSYLSLTPEQWKSHRSYSCQVTHEGSTVEKTVAPTECS